European Patent Specification EP 3 502 128 B1, published November 13, 2024. Title: Epitope. Applicant: HOYU CO., LTD. Application EP. The sequence listing filed with the application follows.

SEQUENCE LISTING (52 sequences)

SEQ ID NO: 1 - protein, 7 aa, Artificial Sequence
  epitope
  misc_feature (1)..(1): Xaa can be any amino acid
  misc_feature (3)..(3): Xaa can be any amino acid
  misc_feature (5)..(6): Xaa can be any amino acid
XEXPXXQ

SEQ ID NO: 2 - protein, 7 aa, Artificial Sequence
  epitope
  misc_feature (3)..(3): Xaa can be any amino acid
  misc_feature (5)..(6): Xaa can be any amino acid
QEXPXXQ

SEQ ID NO: 3 - protein, 7 aa, Artificial Sequence
  epitope
  misc_feature (3)..(3): Xaa can be any amino acid
  misc_feature (5)..(5): Xaa can be any amino acid
QEXPXQQ

SEQ ID NO: 4 - protein, 8 aa, Artificial Sequence
  epitope
  misc_feature (2)..(2): Xaa can be any amino acid
  misc_feature (4)..(4): Xaa can be any amino acid
  misc_feature (6)..(7): Xaa can be any amino acid
QXEXPXXQ

SEQ ID NO: 5 - protein, 10 aa, Artificial Sequence
  epitope
  misc_feature (4)..(4): Xaa can be any amino acid
  misc_feature (6)..(6): Xaa can be any amino acid
  misc_feature (8)..(9): Xaa can be any amino acid
FPQXEXPXXQ

SEQ ID NO: 6 - protein, 15 aa, Artificial Sequence
  epitope
QQFPQQEFPQQQQFP

SEQ ID NO: 7 - protein, 15 aa, Artificial Sequence
  epitope
QQFPQQEAPQQQQFP

SEQ ID NO: 8 - protein, 8 aa, Artificial Sequence
  epitope
  misc_feature (2)..(2): Xaa can be any amino acid
  misc_feature (4)..(5): Xaa can be any amino acid
PXQXXPQQ

SEQ ID NO: 9 - protein, 8 aa, Artificial Sequence
  epitope
  misc_feature (4)..(5): Xaa can be any amino acid
PQQXXPQQ

SEQ ID NO: 10 - protein, 9 aa, Artificial Sequence
  epitope
  misc_feature (3)..(3): Xaa can be any amino acid
  misc_feature (5)..(6): Xaa can be any amino acid
FPXQXXPQQ

SEQ ID NO: 11 - protein, 9 aa, Artificial Sequence
  epitope
  misc_feature (2)..(2): Xaa can be any amino acid
  misc_feature (4)..(5): Xaa can be any amino acid
PXQXXPQQH

SEQ ID NO: 12 - protein, 10 aa, Artificial Sequence
  epitope
  misc_feature (3)..(3): Xaa can be any amino acid
  misc_feature (5)..(6): Xaa can be any amino acid
FPXQXXPQQH

SEQ ID NO: 13 - protein, 15 aa, Artificial Sequence
  epitope
PQQQPPQQHQFPQQQ

SEQ ID NO: 14 - protein, 15 aa, Artificial Sequence
  epitope
PQQQAPQQHQFPQQQ

SEQ ID NO: 15 - protein, 25 aa, Artificial Sequence
  epitope candidate
QFPQQQFPQQEFPQQQQFPQQQIAR

SEQ ID NO: 16 - protein, 10 aa, Artificial Sequence
  epitope candidate
EFPQQQQFPQ

SEQ ID NO: 17 - protein, 10 aa, Artificial Sequence
  epitope candidate
QEFPQQQQFP

SEQ ID NO: 18 - protein, 10 aa, Artificial Sequence
  epitope candidate
QQEFPQQQQF

SEQ ID NO: 19 - protein, 10 aa, Artificial Sequence
  epitope candidate
PQQEFPQQQQ

SEQ ID NO: 20 - protein, 10 aa, Artificial Sequence
  epitope candidate
FPQQEFPQQQ

SEQ ID NO: 21 - protein, 10 aa, Artificial Sequence
  epitope candidate
QFPQQEFPQQ

SEQ ID NO: 22 - protein, 7 aa, Artificial Sequence
  epitope
QEFPQQQ

SEQ ID NO: 23 - protein, 24 aa, Artificial Sequence
  epitope candidate
QFLQQQQFPQQQPPQQHQFPQQQL

SEQ ID NO: 24 - protein, 10 aa, Artificial Sequence
  epitope candidate
QQQPPQQHQF

SEQ ID NO: 25 - protein, 10 aa, Artificial Sequence
  epitope candidate
PQQQPPQQHQ

SEQ ID NO: 26 - protein, 10 aa, Artificial Sequence
  epitope candidate
FPQQQPPQQH

SEQ ID NO: 27 - protein, 10 aa, Artificial Sequence
  epitope candidate
QFPQQQPPQQ

SEQ ID NO: 28 - protein, 10 aa, Artificial Sequence
  epitope candidate
QQFPQQQPPQ

SEQ ID NO: 29 - protein, 8 aa, Artificial Sequence
  epitope
PQQQPPQQ

SEQ ID NO: 30 - protein, 15 aa, Artificial Sequence
  modified epitope
QQFPQQEFPQQAQFP

SEQ ID NO: 31 - protein, 15 aa, Artificial Sequence
  modified epitope
QQFPQQEFPQAQQFP

SEQ ID NO: 32 - protein, 15 aa, Artificial Sequence
  modified epitope
QQFPQQEFPAQQQFP

SEQ ID NO: 33 - protein, 15 aa, Artificial Sequence
  modified epitope
QQFPQQEFAQQQQFP

SEQ ID NO: 34 - protein, 15 aa, Artificial Sequence
  modified epitope
QQFPQQAFPQQQQFP

SEQ ID NO: 35 - protein, 15 aa, Artificial Sequence
  modified epitope
QQFPQAEFPQQQQFP

SEQ ID NO: 36 - protein, 15 aa, Artificial Sequence
  modified epitope
PQQQPPQAHQFPQQQ

SEQ ID NO: 37 - protein, 15 aa, Artificial Sequence
  modified epitope
PQQQPPAQHQFPQQQ

SEQ ID NO: 38 - protein, 15 aa, Artificial Sequence
  modified epitope
PQQQPAQQHQFPQQQ

SEQ ID NO: 39 - protein, 15 aa, Artificial Sequence
  modified epitope
PQQAPPQQHQFPQQQ

SEQ ID NO: 40 - protein, 15 aa, Artificial Sequence
  modified epitope
PQAQPPQQHQFPQQQ

SEQ ID NO: 41 - protein, 15 aa, Artificial Sequence
  modified epitope
PAQQPPQQHQFPQQQ

SEQ ID NO: 42 - protein, 15 aa, Artificial Sequnece
  modified epitope
AQQQPPQQHQFPQQQ

SEQ ID NO: 43 - protein, 7 aa, Artificial Sequence
  known epitope
QQIPQQQ

SEQ ID NO: 44 - protein, 7 aa, Artificial Sequence
  known epitope
QQLPQQQ

SEQ ID NO: 45 - protein, 7 aa, Artificial Sequence
  known epitope
QQFPQQQ

SEQ ID NO: 46 - protein, 8 aa, Artificial Sequence
  epitope
QQEFPQQQ

SEQ ID NO: 47 - protein, 10 aa, Artificial Sequence
  epitope
FPQQEFPQQQ

SEQ ID NO: 48 - protein, 9 aa, Artificial Sequence
  epitope
FPQQQPPQQ

SEQ ID NO: 49 - protein, 9 aa, Artificial Sequence
  epitope
PQQQPPQQH

SEQ ID NO: 50 - protein, 10 aa, Artificial Sequence
  epitope
FPQQQPPQQH

SEQ ID NO: 51 - protein, 439 aa, Triticum aestivum
MKTFIIFVLLAMAMNIASASRLLSPRGKELHTPQEQFPQQQQFPQPQQFPQQQIPQQHQIPQQPQQFPQQQQFLQQQQIPQQQIPQQHQIPQQPQQFPQQQQFPQQHQSPQQQFPQQQFPQQKLPQQEFPQQQISQQPQQLPQQQQIPQQPQQFLQQQQFPQQQPPQQHQFPQQQLPQQQQIPQQQQIPQQPQQIPQQQQIPQQPQQFPQQQFPQQQFPQQQFPQQEFPQQQQFPQQQIARQPQQLPQQQQIPQQPQQFPQQQQFPQQQSPQQQQFPQQQFPQQQQLPQKQFPQPQQIPQQQQIPQQPQQFPQQQFPQQQQFPQQQEFPQQQFPQQQFHQQQLPQQQFPQQQFPQQQFPQQQQFPQQQQLTQQQFPRPQQSPEQQQFPQQQFPQQPPQQFPQQQFPIPYPPQQSEEPSPYQQYPQQQPSGSDVISISGL

SEQ ID NO: 52 - DNA, 1320 bp, Triticum aestivum
atgaagaccttcatcatatttgtcctccttgccatggcgatgaacatcgccagtgccagtaggctgctaagccctagaggcaaggaattgcatactccacaagaacaattcccccaacaacaacaattcccccaaccacaacaattcccccaacaacaaatcccccaacaacatcaaatcccccagcaaccacaacaattcccccaacaacaacaattcctccaacaacaacaaatcccgcaacaacaaatcccccaacaacatcaaatcccccagcaaccacaacaattcccccagcaacagcaattcccccaacaacaccaatccccccaacaacaattcccacaacaacaattcccccaacagaaattgccgcaacaggaattcccacaacaacaaatctcccagcaaccacaacaactcccccagcaacaacaaatcccccagcaaccacaacaatttctccaacaacaacaattcccccagcaacaacccccccaacaacatcaatttccccaacagcaattgccccaacaacaacaaatcccccaacaacaacagatcccccagcaaccacaacaaatcccccaacaacaacaaatcccccagcaaccacaacaattcccccaacaacaattcccgcaacaacaatttccccaacagcaattcccgcaacaggaattcccacaacaacaacaattcccgcaacaacaaatcgcccggcaaccacaacaactcccccaacaacaacaaatcccccagcaaccacaacaatttccccaacaacaacaattcccccagcaacaatcaccccaacaacagcaatttccccaacaacaattcccccaacaacaacaattaccgcaaaaacaattcccccaaccacaacaaataccccaacaacaacaaatcccccagcaaccacaacaattcccccagcaacaattcccccaacaacagcaatttccccaacaacaagaattcccccaacagcaattcccgcaacaacaattccaccaacaacaattaccgcaacaacaatttccccaacaacaattcccccaacagcaattcccccaacaacaacagttcccccaacaacaacaattaacgcaacaacaattcccccggccacaacaatcccctgaacaacaacaattcccccaacaacaattcccccagcaaccaccacaacaattcccccaacaacaatttccaataccatacccaccccagcaatcagaagaaccttccccataccaacaatatccacaacaacaaccatctgggagcgacgttataagtatcagtggcctatga